European Patent Application EP 4 349 997 A2, published April 10, 2024. Title: ANTI-GARP ANTIBODY. Applicant: Daiichi Sankyo Company, Limited. Application EP. The sequence listing filed with the application follows.

SEQUENCE LISTING (57 sequences)

SEQ ID NO: 1 - protein, 662 aa, Homo sapiens
MRPQILLLLALLTLGLAAQHQDKVPCKMVDKKVSCQVLGLLQVPSVLPPDTETLDLSGNQLRSILASPLGFYTALRHLDLSTNEISFLQPGAFQALTHLEHLSLAHNRLAMATALSAGGLGPLPRVTSLDLSGNSLYSGLLERLLGEAPSLHTLSLAENSLTRLTRHTFRDMPALEQLDLHSNVLMDIEDGAFEGLPRLTHLNLSRNSLTCISDFSLQQLRVLDLSCNSIEAFQTASQPQAEFQLTWLDLRENKLLHFPDLAALPRLIYLNLSNNLIRLPTGPPQDSKGIHAPSEGWSALPLSAPSGNASGRPLSQLLNLDLSYNEIELIPDSFLEHLTSLCFLNLSRNCLRTFEARRLGSLPCLMLLDLSHNALETLELGARALGSLRTLLLQGNALRDLPPYTFANLASLQRLNLQGNRVSPCGGPDEPGPSGCVAFSGITSLRSLSLVDNEIELLRAGAFLHTPLTELDLSSNPGLEVATGALGGLEASLEVLALQGNGLMVLQVDLPCFICLKRLNLAENRLSHLPAWTQAVSLEVLDLRNNSFSLLPGSAMGGLETSLRRLYLQGNPLSCCGNGWLAAQLHQGRVDVDATQDLICRFSSQEEVSLSHVRPEDCEKGGLKNINLIIILTFILVSAILLTTLAACCCVRRQKFNQQYKA

SEQ ID NO: 2 - protein, 448 aa, Homo sapiens
EVQLLESGGGLVQPGGSLRLSCAASGFTFSDYYMSWIRQAPGKGLEWVSGVSWNGSRTHYADSVKGRFTISRDNSKNTLYLQMNSLRAEDTAVYYCARQRQLAEFDYWGQGTLVTVSSASTKGPSVFPLAPSSKSTSGGTAALGCLVKDYFPEPVTVSWNSGALTSGVHTFPAVLQSSGLYSLSSVVTVPSSSLGTQTYICNVNHKPSNTKVDKRVEPKSCDKTHTCPPCPAPELLGGPSVFLFPPKPKDTLMISRTPEVTCVVVDVSHEDPEVKFNWYVDGVEVHNAKTKPREEQYNSTYRVVSVLTVLHQDWLNGKEYKCKVSNKALPAPIEKTISKAKGQPREPQVYTLPPSREEMTKNQVSLTCLVKGFYPSDIAVEWESNGQPENNYKTTPPVLDSDGSFFLYSKLTVDKSRWQQGNVFSCSVMHEALHNHYTQKSLSLSPGK

SEQ ID NO: 3 - protein, 217 aa, Homo sapiens
QSVLTQPPSASGTPGQRVTISCTGSSSNIGAGYVVHWYQQLPGTAPKLLIYADTNRPSGVPDRFSGSKSGTSASLAISGLRSEDEADYYCQSYDSSLRGWVFGGGTKLTVLGQPKAAPSVTLFPPSSEELQANKATLVCLISDFYPGAVTVAWKADSSPVKAGVETTTPSKQSNNKYAASSYLSLTPEQWKSHRSYSCQVTHEGSTVEKTVAPTECS

SEQ ID NO: 4 - protein, 453 aa, Homo sapiens
EVQLLESGGGLVQPGGSLRLSCAASGFTFSSYGMHWVRQAPGKGLEWVAGISWNSAITVYADSVKGRFTISRDNSKNTLYLQMNSLRAEDTAVYYCAKDAGGRYSGSYYFDYWGQGTLVTVSSASTKGPSVFPLAPSSKSTSGGTAALGCLVKDYFPEPVTVSWNSGALTSGVHTFPAVLQSSGLYSLSSVVTVPSSSLGTQTYICNVNHKPSNTKVDKRVEPKSCDKTHTCPPCPAPELLGGPSVFLFPPKPKDTLMISRTPEVTCVVVDVSHEDPEVKFNWYVDGVEVHNAKTKPREEQYNSTYRVVSVLTVLHQDWLNGKEYKCKVSNKALPAPIEKTISKAKGQPREPQVYTLPPSREEMTKNQVSLTCLVKGFYPSDIAVEWESNGQPENNYKTTPPVLDSDGSFFLYSKLTVDKSRWQQGNVFSCSVMHEALHNHYTQKSLSLSPGK

SEQ ID NO: 5 - protein, 216 aa, Homo sapiens
QSVLTQPPSASGTPGQRVTISCTGSSSNIGAGYDVHWYQQLPGTAPKLLIYGNSNRPSGVPDRFSGSKSGTSASLAISGLRSEDEADYYCQSYDRSLNWVFGGGTKLTVLGQPKAAPSVTLFPPSSEELQANKATLVCLISDFYPGAVTVAWKADSSPVKAGVETTTPSKQSNNKYAASSYLSLTPEQWKSHRSYSCQVTHEGSTVEKTVAPTECS

SEQ ID NO: 6 - DNA, 1344 bp, Homo sapiens
  source 1..1344: mol_type = other DNA
gaggtgcagctgttggagtctgggggaggcttggtacagcctggggggtccctgagactctcctgtgcagcctctggattcaccttcagtgactactacatgagctggatccgccaggctccaggcaaggggctggagtgggtatcgggtgttagttggaatggcagtaggacgcactatgcagactctgtgaagggccgattcaccatctccagagacaattccaagaacacgctgtatctgcaaatgaacagcctgagagccgaggacactgccgtgtattactgtgccagacagaggcagctggctgaatttgactactggggccaaggtaccctggtcaccgtgagctcagcctccaccaagggcccaagcgtcttccccctggcaccctcctccaagagcacctctggcggcacagccgccctgggctgcctggtcaaggactacttccccgaacccgtgaccgtgagctggaactcaggcgccctgaccagcggcgtgcacaccttccccgctgtcctgcagtcctcaggactctactccctcagcagcgtggtgaccgtgccctccagcagcttgggcacccagacctacatctgcaacgtgaatcacaagcccagcaacaccaaggtggacaagagagttgagcccaaatcttgtgacaaaactcacacatgcccaccctgcccagcacctgaactcctggggggaccctcagtcttcctcttccccccaaaacccaaggacaccctcatgatctcccggacccctgaggtcacatgcgtggtggtggacgtgagccacgaagaccctgaggtcaagttcaactggtacgtggacggcgtggaggtgcataatgccaagacaaagccccgggaggagcagtacaacagcacgtaccgggtggtcagcgtcctcaccgtcctgcaccaggactggctgaatggcaaggagtacaagtgcaaggtctccaacaaagccctcccagcccccatcgagaaaaccatctccaaagccaaaggccagccccgggaaccacaggtgtacaccctgcccccatcccgggaggagatgaccaagaaccaggtcagcctgacctgcctggtcaaaggcttctatcccagcgacatcgccgtggagtgggagagcaatggccagcccgagaacaactacaagaccacccctcccgtgctggactccgacggctccttcttcctctacagcaagctcaccgtggacaagagcaggtggcagcagggcaacgtcttctcatgctccgtgatgcatgaggctctgcacaaccactacacccagaagagcctctccctgtctcccggcaaa

SEQ ID NO: 7 - DNA, 651 bp, Homo sapiens
  source 1..651: mol_type = other DNA
cagtctgtgctgactcagccaccctcagcgtctgggacccccgggcagagggtcaccatctcctgcactgggagcagctccaacattggggcgggttatgttgtacattggtatcagcagctcccaggaacggcccccaaactcctcatctatgctgacaccaatcggccctcaggggtccctgaccgattctctggctccaagtctggcacctcagcctccctggccatcagtgggctccggtccgaggatgaggctgattattactgccagtcctatgacagcagcctgagaggttgggtgttcggcggaggaaccaagctgacggtcctaggtcagcctaaggctgcccctagcgtgaccctgttccctccttccagcgaggagcttcaagctaacaaggccaccctggtgtgtcttatctctgacttctaccctggcgctgtgaccgtggcctggaaggctgacagctcccctgtgaaggccggagtggagaccaccacacctagcaagcagtctaacaacaagtacgctgccagctcctacctgagccttacccctgagcagtggaagtctcacagaagctactcctgtcaagtgacccacgagggcagcaccgtggagaagaccgtggctcctaccgagtgttcc

SEQ ID NO: 8 - DNA, 1359 bp, Homo sapiens
  source 1..1359: mol_type = other DNA
gaggtgcagctgttggagtctgggggaggcttggtacagcctggggggtccctgagactctcctgtgcagcctctggattcaccttcagtagctatggcatgcactgggtccgccaggctccaggcaaggggctggagtgggtcgccggaattagttggaacagtgccatcacagtctatgcggactctgtgaagggccggttcaccatctccagagacaattccaagaacacgctgtatctgcaaatgaacagcctgagagccgaggacactgccgtgtattactgtgcaaaagatgccgggggccggtatagtgggagctactactttgactactggggccaaggtaccctggtcaccgtgagctcagcctccaccaagggcccaagcgtcttccccctggcaccctcctccaagagcacctctggcggcacagccgccctgggctgcctggtcaaggactacttccccgaacccgtgaccgtgagctggaactcaggcgccctgaccagcggcgtgcacaccttccccgctgtcctgcagtcctcaggactctactccctcagcagcgtggtgaccgtgccctccagcagcttgggcacccagacctacatctgcaacgtgaatcacaagcccagcaacaccaaggtggacaagagagttgagcccaaatcttgtgacaaaactcacacatgcccaccctgcccagcacctgaactcctggggggaccctcagtcttcctcttccccccaaaacccaaggacaccctcatgatctcccggacccctgaggtcacatgcgtggtggtggacgtgagccacgaagaccctgaggtcaagttcaactggtacgtggacggcgtggaggtgcataatgccaagacaaagccccgggaggagcagtacaacagcacgtaccgggtggtcagcgtcctcaccgtcctgcaccaggactggctgaatggcaaggagtacaagtgcaaggtctccaacaaagccctcccagcccccatcgagaaaaccatctccaaagccaaaggccagccccgggaaccacaggtgtacaccctgcccccatcccgggaggagatgaccaagaaccaggtcagcctgacctgcctggtcaaaggcttctatcccagcgacatcgccgtggagtgggagagcaatggccagcccgagaacaactacaagaccacccctcccgtgctggactccgacggctccttcttcctctacagcaagctcaccgtggacaagagcaggtggcagcagggcaacgtcttctcatgctccgtgatgcatgaggctctgcacaaccactacacccagaagagcctctccctgtctcccggcaaa

SEQ ID NO: 9 - DNA, 648 bp, Homo sapiens
  source 1..648: mol_type = other DNA
cagtctgtgctgactcagccaccctcagcgtctgggacccccgggcagagggtcaccatctcctgcactgggagcagctccaacatcggggcaggttatgatgtacactggtatcagcagctcccaggaacggcccccaaactcctcatctatggtaacagcaatcggccctcaggggtccctgaccgattctctggctccaagtctggcacctcagcctccctggccatcagtgggctccggtccgaggatgaggctgattattactgccagtcctatgacagaagcctgaattgggtgttcggcggaggaaccaagctgacggtcctaggtcagcctaaggctgcccctagcgtgaccctgttccctccttccagcgaggagcttcaagctaacaaggccaccctggtgtgtcttatctctgacttctaccctggcgctgtgaccgtggcctggaaggctgacagctcccctgtgaaggccggagtggagaccaccacacctagcaagcagtctaacaacaagtacgctgccagctcctacctgagccttacccctgagcagtggaagtctcacagaagctactcctgtcaagtgacccacgagggcagcaccgtggagaagaccgtggctcctaccgagtgttcc

SEQ ID NO: 10 - DNA, 24 bp, synthetic construct
  misc_feature 1..24: note = Primer A
  source 1..24: mol_type = other DNA
gaaacagctatgaaatacctattg

SEQ ID NO: 11 - DNA, 19 bp, synthetic construct
  misc_feature 1..19: note = Primer B
  source 1..19: mol_type = other DNA
gcctgagcagtggaagtcc

SEQ ID NO: 12 - DNA, 24 bp, synthetic construct
  misc_feature 1..24: note = Primer C
  source 1..24: mol_type = other DNA
taggtatttcattatgactgtctc

SEQ ID NO: 13 - DNA, 23 bp, synthetic construct
  misc_feature 1..23: note = Primer D
  source 1..23: mol_type = other DNA
cccagtcacgacgttgtaaaacg

SEQ ID NO: 14 - DNA, 351 bp, Rattus rattus
  source 1..351: mol_type = other DNA
gaggtgcagctggtggagtctgggggaggcttagtgcagcctggaaggtccaagaaactctcctgttcagcctcaggattcactttcagtaactattacatggcctgggtccgccaggctccaacgcagggtctggagtgggtcgcatccattggtactgttggtggtaacacttactatcgagactccgtgaagggccgattcactatctccagagatgatgcaaaaagcaccctatacctgcaaatggacagtctgaggtctgaggacacggccacttattactgtgcaagagaggattacggagggtttccccactggggccaaggagtcatggtcacagtctcctca

SEQ ID NO: 15 - protein, 117 aa, Rattus rattus
EVQLVESGGGLVQPGRSKKLSCSASGFTFSNYYMAWVRQAPTQGLEWVASIGTVGGNTYYRDSVKGRFTISRDDAKSTLYLQMDSLRSEDTATYYCAREDYGGFPHWGQGVMVTVSS

SEQ ID NO: 16 - DNA, 327 bp, Rattus rattus
  source 1..327: mol_type = other DNA
aatattgtgatgactcagtctcccacatccatgttcatatcagtcggagacagggtcaccatgaactgtaaggccagtcagaatgtgggaactaatgtagactggtaccagcagaaaacagggcagtctcctaaactgcttatctatggggcgtccaaccgctacactggagtccctgatcgcttcacaggcagtggatctggaacagatttcactctcaccatcagcaacatgcaggctgaagacctggctgtttatgactgtctacagtataagtacaatccatacacgtttggaactgggaccaagctggaactgaaccgggct

SEQ ID NO: 17 - protein, 109 aa, Rattus rattus
NIVMTQSPTSMFISVGDRVTMNCKASQNVGTNVDWYQQKTGQSPKLLIYGASNRYTGVPDRFTGSGSGTDFTLTISNMQAEDLAVYDCLQYKYNPYTFGTGTKLELNRA

SEQ ID NO: 18 - DNA, 360 bp, Rattus rattus
  source 1..360: mol_type = other DNA
caggtgcagctgagggagtcaggacctggtctggtgcagccctcacagaccctgtccctcacctgcactgtctctgggttctcactaaccagctttcatgtaagctgggttcgccagcctccagagaagggtctggagtggattgcaacaatttcaagtggtggaggtacatattataattcagctctcaaatcccgactgagcatcagcagggacacctccaagagccaagttttcttaaagatgagcactctgcaaactgaagacacagccatgtacttctgtgcccggatttcgggctggggccattactatgttatggatgtctggggtcaaggagcttcagtcactgtctcctca

SEQ ID NO: 19 - protein, 120 aa, Rattus rattus
QVQLRESGPGLVQPSQTLSLTCTVSGFSLTSFHVSWVRQPPEKGLEWIATISSGGGTYYNSALKSRLSISRDTSKSQVFLKMSTLQTEDTAMYFCARISGWGHYYVMDVWGQGASVTVSS

SEQ ID NO: 20 - DNA, 327 bp, Rattus rattus
  source 1..327: mol_type = other DNA
gacatccagatgacacagtctccagcttccctgtctggatctctgggagaaactgtcaccatccaatgtcaagcaagtgaggacatttacagtggtttagcgtggtatcagcagaagccagggaaatctcctcagctcctgatctatggtgcaggtagcttacaagacggcgtcccatcacgattcagtggcggtggatctggcacacattattctctcaagatcagcagcatgcaaactgaagatgaaggggtttatttctgtcaacagggtttaaagtttccgctcacgttcggttctgggaccaagctggagatcaaacgggct

SEQ ID NO: 21 - protein, 109 aa, Rattus rattus
DIQMTQSPASLSGSLGETVTIQCQASEDIYSGLAWYQQKPGKSPQLLIYGAGSLQDGVPSRFSGGGSGTHYSLKISSMQTEDEGVYFCQQGLKFPLTFGSGTKLEIKRA

SEQ ID NO: 22 - DNA, 449 bp, Homo sapiens
  source 1..449: mol_type = other DNA
gcctccggactctagagccaccatggtgctgcagacccaggtgttcatctccctgctgctgtggatctccggcgcgtacggcgatatcgtgatgattaaacgtacggtggccgccccctccgtgttcatcttccccccctccgacgagcagctgaagtccggcaccgcctccgtggtgtgcctgctgaataacttctaccccagagaggccaaggtgcagtggaaggtggacaacgccctgcagtccgggaactcccaggagagcgtgaccgagcaggacagcaaggacagcacctacagcctgagcagcaccctgaccctgagcaaagccgactacgagaagcacaaggtgtacgcctgcgaggtgacccaccagggcctgagctcccccgtcaccaagagcttcaacaggggggagtgttaggggcccgtttaaacgggggaggcta

SEQ ID NO: 23 - DNA, 1132 bp, Homo sapiens
  source 1..1132: mol_type = other DNA
gcctccggactctagagccaccatgaaacacctgtggttcttcctcctgctggtggcagctcccagatgggtgctgagccaggtgcaattgtgcaggcggttagctcagcctccaccaagggcccaagcgtcttccccctggcaccctcctccaagagcacctctggcggcacagccgccctgggctgcctggtcaaggactacttccccgaacccgtgaccgtgagctggaactcaggcgccctgaccagcggcgtgcacaccttccccgctgtcctgcagtcctcaggactctactccctcagcagcgtggtgaccgtgccctccagcagcttgggcacccagacctacatctgcaacgtgaatcacaagcccagcaacaccaaggtggacaagagagttgagcccaaatcttgtgacaaaactcacacatgcccaccctgcccagcacctgaactcctggggggaccctcagtcttcctcttccccccaaaacccaaggacaccctcatgatctcccggacccctgaggtcacatgcgtggtggtggacgtgagccacgaagaccctgaggtcaagttcaactggtacgtggacggcgtggaggtgcataatgccaagacaaagccccgggaggagcagtacaacagcacgtaccgggtggtcagcgtcctcaccgtcctgcaccaggactggctgaatggcaaggagtacaagtgcaaggtctccaacaaagccctcccagcccccatcgagaaaaccatctccaaagccaaaggccagccccgggaaccacaggtgtacaccctgcccccatcccgggaggagatgaccaagaaccaggtcagcctgacctgcctggtcaaaggcttctatcccagcgacatcgccgtggagtgggagagcaatggccagcccgagaacaactacaagaccacccctcccgtgctggactccgacggctccttcttcctctacagcaagctcaccgtggacaagagcaggtggcagcagggcaacgtcttctcatgctccgtgatgcatgaggctctgcacaaccactacacccagaagagcctctccctgtctcccggcaaatgagatatcgggcccgtttaaacgggggaggcta

SEQ ID NO: 24 - DNA, 1398 bp, synthetic construct
  misc_feature 1..1398: note = Chimeric Antibody
  source 1..1398: mol_type = other DNA
atgaaacacctgtggttcttcctcctgctggtggcagctcccagatgggtgctgagcgaggtgcagctggtggagtctgggggaggcttagtgcagcctggaaggtccaagaaactctcctgttcagcctcaggattcactttcagtaactattacatggcctgggtccgccaggctccaacgcagggtctggagtgggtcgcatccattggtactgttggtggtaacacttactatcgagactccgtgaagggccgattcactatctccagagatgatgcaaaaagcaccctatacctgcaaatggacagtctgaggtctgaggacacggccacttattactgtgcaagagaggattacggagggtttccccactggggccaaggagtcatggtcacagtcagctcagcctccaccaagggcccaagcgtcttccccctggcaccctcctccaagagcacctctggcggcacagccgccctgggctgcctggtcaaggactacttccccgaacccgtgaccgtgagctggaactcaggcgccctgaccagcggcgtgcacaccttccccgctgtcctgcagtcctcaggactctactccctcagcagcgtggtgaccgtgccctccagcagcttgggcacccagacctacatctgcaacgtgaatcacaagcccagcaacaccaaggtggacaagagagttgagcccaaatcttgtgacaaaactcacacatgcccaccctgcccagcacctgaactcctggggggaccctcagtcttcctcttccccccaaaacccaaggacaccctcatgatctcccggacccctgaggtcacatgcgtggtggtggacgtgagccacgaagaccctgaggtcaagttcaactggtacgtggacggcgtggaggtgcataatgccaagacaaagccccgggaggagcagtacaacagcacgtaccgggtggtcagcgtcctcaccgtcctgcaccaggactggctgaatggcaaggagtacaagtgcaaggtctccaacaaagccctcccagcccccatcgagaaaaccatctccaaagccaaaggccagccccgggaaccacaggtgtacaccctgcccccatcccgggaggagatgaccaagaaccaggtcagcctgacctgcctggtcaaaggcttctatcccagcgacatcgccgtggagtgggagagcaatggccagcccgagaacaactacaagaccacccctcccgtgctggactccgacggctccttcttcctctacagcaagctcaccgtggacaagagcaggtggcagcagggcaacgtcttctcatgctccgtgatgcatgaggctctgcacaaccactacacccagaagagcctctccctgtctcccggcaaa

SEQ ID NO: 25 - protein, 466 aa, synthetic construct
  REGION 1..466: note = Chimeric Antibody
MKHLWFFLLLVAAPRWVLSEVQLVESGGGLVQPGRSKKLSCSASGFTFSNYYMAWVRQAPTQGLEWVASIGTVGGNTYYRDSVKGRFTISRDDAKSTLYLQMDSLRSEDTATYYCAREDYGGFPHWGQGVMVTVSSASTKGPSVFPLAPSSKSTSGGTAALGCLVKDYFPEPVTVSWNSGALTSGVHTFPAVLQSSGLYSLSSVVTVPSSSLGTQTYICNVNHKPSNTKVDKRVEPKSCDKTHTCPPCPAPELLGGPSVFLFPPKPKDTLMISRTPEVTCVVVDVSHEDPEVKFNWYVDGVEVHNAKTKPREEQYNSTYRVVSVLTVLHQDWLNGKEYKCKVSNKALPAPIEKTISKAKGQPREPQVYTLPPSREEMTKNQVSLTCLVKGFYPSDIAVEWESNGQPENNYKTTPPVLDSDGSFFLYSKLTVDKSRWQQGNVFSCSVMHEALHNHYTQKSLSLSPGK

SEQ ID NO: 26 - DNA, 702 bp, synthetic construct
  misc_feature 1..702: note = Chimeric Antibody
  source 1..702: mol_type = other DNA
atggtgctgcagacccaggtgttcatctccctgctgctgtggatctccggcgcgtacggcaatattgtgatgactcagtctcccacatccatgttcatatcagtcggagacagggtcaccatgaactgtaaggccagtcagaatgtgggaactaatgtagactggtaccagcagaaaacagggcagtctcctaaactgcttatctatggggcgtccaaccgctacactggagtccctgatcgcttcacaggcagtggatctggaacagatttcactctcaccatcagcaacatgcaggctgaagacctggctgtttatgactgtctacagtataagtacaatccatacacgtttggaactgggaccaagctggaactgaaccgggctgtggccgccccctccgtgttcatcttccccccctccgacgagcagctgaagtccggcaccgcctccgtggtgtgcctgctgaataacttctaccccagagaggccaaggtgcagtggaaggtggacaacgccctgcagtccgggaactcccaggagagcgtgaccgagcaggacagcaaggacagcacctacagcctgagcagcaccctgaccctgagcaaagccgactacgagaagcacaaggtgtacgcctgcgaggtgacccaccagggcctgagctcccccgtcaccaagagcttcaacaggggggagtgt

SEQ ID NO: 27 - protein, 234 aa, synthetic construct
  REGION 1..234: note = Chimeric Antibody
MVLQTQVFISLLLWISGAYGNIVMTQSPTSMFISVGDRVTMNCKASQNVGTNVDWYQQKTGQSPKLLIYGASNRYTGVPDRFTGSGSGTDFTLTISNMQAEDLAVYDCLQYKYNPYTFGTGTKLELNRAVAAPSVFIFPPSDEQLKSGTASVVCLLNNFYPREAKVQWKVDNALQSGNSQESVTEQDSKDSTYSLSSTLTLSKADYEKHKVYACEVTHQGLSSPVTKSFNRGEC

SEQ ID NO: 28 - DNA, 1407 bp, synthetic construct
  misc_feature 1..1407: note = Chimeric Antibody
  source 1..1407: mol_type = other DNA
atgaaacacctgtggttcttcctcctgctggtggcagctcccagatgggtgctgagccaggtgcagctgagggagtcaggacctggtctggtgcagccctcacagaccctgtccctcacctgcactgtctctgggttctcactaaccagctttcatgtaagctgggttcgccagcctccagagaagggtctggagtggattgcaacaatttcaagtggtggaggtacatattataattcagctctcaaatcccgactgagcatcagcagggacacctccaagagccaagttttcttaaagatgagcactctgcaaactgaagacacagccatgtacttctgtgcccggatttcgggctggggccattactatgttatggatgtctggggtcaaggagcttcagtcactgtcagctcagcctccaccaagggcccaagcgtcttccccctggcaccctcctccaagagcacctctggcggcacagccgccctgggctgcctggtcaaggactacttccccgaacccgtgaccgtgagctggaactcaggcgccctgaccagcggcgtgcacaccttccccgctgtcctgcagtcctcaggactctactccctcagcagcgtggtgaccgtgccctccagcagcttgggcacccagacctacatctgcaacgtgaatcacaagcccagcaacaccaaggtggacaagagagttgagcccaaatcttgtgacaaaactcacacatgcccaccctgcccagcacctgaactcctggggggaccctcagtcttcctcttccccccaaaacccaaggacaccctcatgatctcccggacccctgaggtcacatgcgtggtggtggacgtgagccacgaagaccctgaggtcaagttcaactggtacgtggacggcgtggaggtgcataatgccaagacaaagccccgggaggagcagtacaacagcacgtaccgggtggtcagcgtcctcaccgtcctgcaccaggactggctgaatggcaaggagtacaagtgcaaggtctccaacaaagccctcccagcccccatcgagaaaaccatctccaaagccaaaggccagccccgggaaccacaggtgtacaccctgcccccatcccgggaggagatgaccaagaaccaggtcagcctgacctgcctggtcaaaggcttctatcccagcgacatcgccgtggagtgggagagcaatggccagcccgagaacaactacaagaccacccctcccgtgctggactccgacggctccttcttcctctacagcaagctcaccgtggacaagagcaggtggcagcagggcaacgtcttctcatgctccgtgatgcatgaggctctgcacaaccactacacccagaagagcctctccctgtctcccggcaaa

SEQ ID NO: 29 - protein, 469 aa, synthetic construct
  REGION 1..469: note = Chimeric Antibody
MKHLWFFLLLVAAPRWVLSQVQLRESGPGLVQPSQTLSLTCTVSGFSLTSFHVSWVRQPPEKGLEWIATISSGGGTYYNSALKSRLSISRDTSKSQVFLKMSTLQTEDTAMYFCARISGWGHYYVMDVWGQGASVTVSSASTKGPSVFPLAPSSKSTSGGTAALGCLVKDYFPEPVTVSWNSGALTSGVHTFPAVLQSSGLYSLSSVVTVPSSSLGTQTYICNVNHKPSNTKVDKRVEPKSCDKTHTCPPCPAPELLGGPSVFLFPPKPKDTLMISRTPEVTCVVVDVSHEDPEVKFNWYVDGVEVHNAKTKPREEQYNSTYRVVSVLTVLHQDWLNGKEYKCKVSNKALPAPIEKTISKAKGQPREPQVYTLPPSREEMTKNQVSLTCLVKGFYPSDIAVEWESNGQPENNYKTTPPVLDSDGSFFLYSKLTVDKSRWQQGNVFSCSVMHEALHNHYTQKSLSLSPGK

SEQ ID NO: 30 - DNA, 702 bp, synthetic construct
  misc_feature 1..702: note = Chimeric Antibody
  source 1..702: mol_type = other DNA
atggtgctgcagacccaggtgttcatctccctgctgctgtggatctccggcgcgtacggcgacatccagatgacacagtctccagcttccctgtctggatctctgggagaaactgtcaccatccaatgtcaagcaagtgaggacatttacagtggtttagcgtggtatcagcagaagccagggaaatctcctcagctcctgatctatggtgcaggtagcttacaagacggcgtcccatcacgattcagtggcggtggatctggcacacattattctctcaagatcagcagcatgcaaactgaagatgaaggggtttatttctgtcaacagggtttaaagtttccgctcacgttcggttctgggaccaagctggagatcaaacgggctgtggccgccccctccgtgttcatcttccccccctccgacgagcagctgaagtccggcaccgcctccgtggtgtgcctgctgaataacttctaccccagagaggccaaggtgcagtggaaggtggacaacgccctgcagtccgggaactcccaggagagcgtgaccgagcaggacagcaaggacagcacctacagcctgagcagcaccctgaccctgagcaaagccgactacgagaagcacaaggtgtacgcctgcgaggtgacccaccagggcctgagctcccccgtcaccaagagcttcaacaggggggagtgt

SEQ ID NO: 31 - protein, 234 aa, synthetic construct
  REGION 1..234: note = Chimeric Antibody
MVLQTQVFISLLLWISGAYGDIQMTQSPASLSGSLGETVTIQCQASEDIYSGLAWYQQKPGKSPQLLIYGAGSLQDGVPSRFSGGGSGTHYSLKISSMQTEDEGVYFCQQGLKFPLTFGSGTKLEIKRAVAAPSVFIFPPSDEQLKSGTASVVCLLNNFYPREAKVQWKVDNALQSGNSQESVTEQDSKDSTYSLSSTLTLSKADYEKHKVYACEVTHQGLSSPVTKSFNRGEC

SEQ ID NO: 32 - DNA, 1398 bp, synthetic construct
  misc_feature 1..1398: note = Humanized Antibody
  source 1..1398: mol_type = other DNA
atgaagcacctgtggttctttctgctgctggtggccgctcccagatgggtgctgtctgaagtgcagctggtggaatccggcggaggcctggtgcagcctggcggatctctgagactgtcttgtgccgcctccggcttcaccttctccaactactacatggcctgggtgcgacaggcccctggcaagggactggaatgggtgtcctctatcggcaccgtgggcggcaacacctactacgccgattctgtgaagggccggttcaccatctcccgggacgactccaagaacaccctgtacctgcagatgaactccctgcgggccgaggacaccgccgtgtactactgtgccagagaggactacggcggcttccctcattggggccagggcacactcgtgaccgtgtcctctgcttccaccaagggcccctccgtgtttcctctggccccttccagcaagtccacctctggcggaacagccgctctgggctgcctcgtgaaggactacttccccgagcccgtgacagtgtcttggaactctggcgccctgacctccggcgtgcacacctttccagctgtgctgcagtcctccggcctgtactccctgtcctccgtcgtgactgtgccctccagctctctgggcacccagacctacatctgcaacgtgaaccacaagccctccaacaccaaggtggacaagcgggtggaacccaagtcctgcgacaagacccacacctgtcccccttgtcctgcccctgaactgctgggcggaccttccgtgttcctgttccccccaaagcctaaggacaccctgatgatctcccggacccccgaagtgacctgcgtggtggtggatgtgtcccacgaggaccctgaagtgaagttcaattggtacgtggacggcgtggaagtgcacaacgccaagaccaagcctagagaggaacagtacaactccacctaccgggtggtgtccgtgctgaccgtgctgcatcaggactggctgaacggcaaagagtacaagtgcaaggtgtccaacaaggccctgcctgcccccatcgaaaagaccatctccaaggccaagggccagccccgggaaccccaggtgtacacactgccccctagccgggaagagatgaccaagaaccaggtgtccctgacctgtctcgtgaaaggcttctacccctccgatatcgccgtggaatgggagagcaacggccagcccgagaacaactacaagaccaccccccctgtgctggactccgacggctcattcttcctgtacagcaagctgacagtggacaagtcccggtggcagcagggcaacgtgttctcctgctccgtgatgcacgaggccctgcacaaccactacacccagaagtccctgtccctgagccccggcaaa

SEQ ID NO: 33 - protein, 466 aa, synthetic construct
  REGION 1..466: note = Humanized Antibody
MKHLWFFLLLVAAPRWVLSEVQLVESGGGLVQPGGSLRLSCAASGFTFSNYYMAWVRQAPGKGLEWVSSIGTVGGNTYYADSVKGRFTISRDDSKNTLYLQMNSLRAEDTAVYYCAREDYGGFPHWGQGTLVTVSSASTKGPSVFPLAPSSKSTSGGTAALGCLVKDYFPEPVTVSWNSGALTSGVHTFPAVLQSSGLYSLSSVVTVPSSSLGTQTYICNVNHKPSNTKVDKRVEPKSCDKTHTCPPCPAPELLGGPSVFLFPPKPKDTLMISRTPEVTCVVVDVSHEDPEVKFNWYVDGVEVHNAKTKPREEQYNSTYRVVSVLTVLHQDWLNGKEYKCKVSNKALPAPIEKTISKAKGQPREPQVYTLPPSREEMTKNQVSLTCLVKGFYPSDIAVEWESNGQPENNYKTTPPVLDSDGSFFLYSKLTVDKSRWQQGNVFSCSVMHEALHNHYTQKSLSLSPGK

SEQ ID NO: 34 - DNA, 1398 bp, synthetic construct
  misc_feature 1..1398: note = Humanized Antibody
  source 1..1398: mol_type = other DNA
atgaagcacctgtggttctttctgctgctggtggccgctcccagatgggtgctgtctgaagtgcagctggtggaatccggcggaggcctggtgcagcctggcggatctctgagactgtcttgtgccgcctccggcttcaccttctccaactactacatggcctgggtgcgacaggcccctggcaagggactggaatgggtggcctctatcggcaccgtgggcggcaacacctactaccgggattctgtgaagggccggttcaccatctcccgggacgactccaagtccaccctgtacctgcagatgaactccctgcgggccgaggacaccgccgtgtactactgtgccagagaggactacggcggcttccctcattggggccagggcacactcgtgaccgtgtcctctgcttccaccaagggcccctccgtgtttcctctggccccttccagcaagtctacctccggcggaacagccgctctgggctgcctcgtgaaggactacttccccgagcccgtgacagtgtcttggaactctggcgccctgaccagcggcgtgcacacctttccagctgtgctgcagtcctccggcctgtactccctgtcctccgtcgtgactgtgccctccagctctctgggcacccagacctacatctgcaacgtgaaccacaagccctccaacaccaaggtggacaagcgggtggaacccaagtcctgcgacaagacccacacctgtcccccttgtcctgcccctgaactgctgggcggaccttccgtgttcctgttccccccaaagcccaaggacaccctgatgatctcccggacccccgaagtgacctgcgtggtggtggatgtgtcccacgaggaccctgaagtgaagttcaattggtacgtggacggcgtggaagtgcacaacgccaagaccaagcctagagaggaacagtacaactccacctaccgggtggtgtccgtgctgaccgtgctgcatcaggactggctgaacggcaaagagtacaagtgcaaggtgtccaacaaggccctgcctgcccccatcgaaaagaccatctccaaggccaagggccagccccgggaaccccaggtgtacacactgccccctagccgggaagagatgaccaagaaccaggtgtccctgacctgtctcgtgaaaggcttctacccctccgatatcgccgtggaatgggagtccaacggccagcctgagaacaactacaagaccaccccccctgtgctggactccgacggctcattcttcctgtacagcaagctgacagtggacaagtcccggtggcagcagggcaacgtgttctcctgctccgtgatgcacgaggccctgcacaaccactacacccagaagtccctgtccctgagccccggcaaa

SEQ ID NO: 35 - protein, 466 aa, synthetic construct
  REGION 1..466: note = Humanized Antibody
MKHLWFFLLLVAAPRWVLSEVQLVESGGGLVQPGGSLRLSCAASGFTFSNYYMAWVRQAPGKGLEWVASIGTVGGNTYYRDSVKGRFTISRDDSKSTLYLQMNSLRAEDTAVYYCAREDYGGFPHWGQGTLVTVSSASTKGPSVFPLAPSSKSTSGGTAALGCLVKDYFPEPVTVSWNSGALTSGVHTFPAVLQSSGLYSLSSVVTVPSSSLGTQTYICNVNHKPSNTKVDKRVEPKSCDKTHTCPPCPAPELLGGPSVFLFPPKPKDTLMISRTPEVTCVVVDVSHEDPEVKFNWYVDGVEVHNAKTKPREEQYNSTYRVVSVLTVLHQDWLNGKEYKCKVSNKALPAPIEKTISKAKGQPREPQVYTLPPSREEMTKNQVSLTCLVKGFYPSDIAVEWESNGQPENNYKTTPPVLDSDGSFFLYSKLTVDKSRWQQGNVFSCSVMHEALHNHYTQKSLSLSPGK

SEQ ID NO: 36 - DNA, 702 bp, synthetic construct
  misc_feature 1..702: note = Humanized Antibody
  source 1..702: mol_type = other DNA
atggtgctgcagacccaggtgttcatctccctgctgctgtggatctccggcgcctacggcaacatcgtgatgacccagtcccccgactccctggctgtgtctctgggcgagagagccaccatcaactgcaaggcctcccagaacgtgggcaccaacgtggactggtatcagcagaagcccggccagtcccctaagctgctgatctacggcgccagcaaccggtacaccggcgtgcccgatagattctccggctctggctctggcaccgactttaccctgacaatcagctctctgcaggccgaggacgtggccgtgtacgactgcctgcagtacaagtacaacccctacaccttcggccagggcacaaaggtggaaatcaagcggaccgtggccgctccctccgtgtttatcttcccaccctccgacgagcagctgaagtccggcacagcttccgtcgtgtgcctgctgaacaacttctacccccgcgaggccaaggtgcagtggaaggtggacaacgccctgcagtccggcaactcccaggaatccgtgaccgagcaggactccaaggacagcacctactccctgtcctccaccctgaccctgtccaaggccgactacgagaagcacaaggtgtacgcctgcgaagtgacccaccagggcctgtctagccccgtgaccaagtctttcaaccggggcgagtgc

SEQ ID NO: 37 - protein, 234 aa, synthetic construct
  REGION 1..234: note = Humanized Antibody
MVLQTQVFISLLLWISGAYGNIVMTQSPDSLAVSLGERATINCKASQNVGTNVDWYQQKPGQSPKLLIYGASNRYTGVPDRFSGSGSGTDFTLTISSLQAEDVAVYDCLQYKYNPYTFGQGTKVEIKRTVAAPSVFIFPPSDEQLKSGTASVVCLLNNFYPREAKVQWKVDNALQSGNSQESVTEQDSKDSTYSLSSTLTLSKADYEKHKVYACEVTHQGLSSPVTKSFNRGEC

SEQ ID NO: 38 - DNA, 702 bp, synthetic construct
  misc_feature 1..702: note = Humanized Antibody
  source 1..702: mol_type = other DNA
atggtgctgcagacccaggtgttcatctccctgctgctgtggatctccggcgcctacggcaacatcgtgatgacccagtccccctccagcctgtctgcttccgtgggcgacagagtgaccatcaactgcaaggcctcccagaacgtgggcaccaacgtggactggtatcagcagaagcccggcaagtcccccaagctgctgatctacggcgccagcaacagatacaccggcgtgcccgacagattctccggctctggctctggcaccgactttaccctgaccatcagctccctgcagcccgaggacttcgccacctacgactgcctgcagtacaagtacaacccctacaccttcggccagggcacaaaggtggaaatcaagcggaccgtggccgctccctccgtgtttatcttcccaccctccgacgagcagctgaagtccggcacagcttctgtcgtgtgcctgctgaacaacttctacccccgcgaggccaaggtgcagtggaaggtggacaacgccctgcagtccggcaactcccaggaatccgtgaccgagcaggactccaaggacagcacctactccctgtcctccaccctgaccctgtccaaggccgactacgagaagcacaaggtgtacgcctgcgaagtgacccaccagggcctgtctagccccgtgaccaagtctttcaaccggggcgagtgc

SEQ ID NO: 39 - protein, 234 aa, synthetic construct
  REGION 1..234: note = Humanized Antibody
MVLQTQVFISLLLWISGAYGNIVMTQSPSSLSASVGDRVTINCKASQNVGTNVDWYQQKPGKSPKLLIYGASNRYTGVPDRFSGSGSGTDFTLTISSLQPEDFATYDCLQYKYNPYTFGQGTKVEIKRTVAAPSVFIFPPSDEQLKSGTASVVCLLNNFYPREAKVQWKVDNALQSGNSQESVTEQDSKDSTYSLSSTLTLSKADYEKHKVYACEVTHQGLSSPVTKSFNRGEC

SEQ ID NO: 40 - DNA, 1407 bp, synthetic construct
  misc_feature 1..1407: note = Humanized Antibody
  source 1..1407: mol_type = other DNA
atgaagcacctgtggttctttctgctgctggtggccgctcccagatgggtgctgtctgaagtgcagctggtggaatccggcggaggcctcgtgaagccttcccagaccctgtctctgacctgcaccgtgtccggcttctccctgacctccttccacgtgtcatgggtgcgacagcctccaggcaagggcctggaatggatcgccaccatctcctctggcggcggaacctactacaaccccagcctgaagtccagagtgaccatctcccgggacacctccaagaaccaggtgtccctgaagctgtcctccgtgaccgccgctgataccgccgtgtactactgcgccagaatctccggctggggccactactacgtgatggacgtgtggggccagggcaccctcgtgacagtgtcctctgcttccaccaagggcccctccgtgtttcctctggccccttccagcaagtctacctccggcggaacagccgctctgggctgcctcgtgaaagactacttccccgagcccgtgaccgtgtcttggaactctggcgctctgaccagcggcgtgcacacctttccagctgtgctgcagtcctccggcctgtactccctgtccagcgtcgtgactgtgccctccagctctctgggcacccagacctacatctgcaacgtgaaccacaagccctccaacaccaaggtggacaagcgggtggaacccaagtcctgcgacaagacccacacctgtcccccttgtcctgcccctgaactgctgggcggaccttccgtgttcctgttccccccaaagcccaaggacaccctgatgatctcccggacccccgaagtgacctgcgtggtggtggatgtgtcccacgaggaccctgaagtgaagttcaattggtacgtggacggcgtggaagtgcacaacgccaagaccaagcctagagaggaacagtacaactccacctaccgggtggtgtccgtgctgaccgtgctgcaccaggattggctgaacggcaaagagtacaagtgcaaggtgtccaacaaggccctgcctgcccccatcgaaaagaccatcagcaaggccaagggccagccccgggaaccccaggtgtacacactgccccctagccgggaagagatgacaaaaaatcaggtgtcactgacctgtctcgtgaagggcttctacccctccgatatcgccgtggaatgggagtccaacggccagcctgagaacaactacaagaccaccccccctgtgctggactccgacggctcattcttcctgtacagcaagctgacagtggacaagtcccggtggcagcagggcaacgtgttctcctgctccgtgatgcacgaggccctgcacaaccactacacccagaagtccctgtccctgagccccggcaaa

SEQ ID NO: 41 - protein, 469 aa, synthetic construct
  REGION 1..469: note = Humanized Antibody
MKHLWFFLLLVAAPRWVLSEVQLVESGGGLVKPSQTLSLTCTVSGFSLTSFHVSWVRQPPGKGLEWIATISSGGGTYYNPSLKSRVTISRDTSKNQVSLKLSSVTAADTAVYYCARISGWGHYYVMDVWGQGTLVTVSSASTKGPSVFPLAPSSKSTSGGTAALGCLVKDYFPEPVTVSWNSGALTSGVHTFPAVLQSSGLYSLSSVVTVPSSSLGTQTYICNVNHKPSNTKVDKRVEPKSCDKTHTCPPCPAPELLGGPSVFLFPPKPKDTLMISRTPEVTCVVVDVSHEDPEVKFNWYVDGVEVHNAKTKPREEQYNSTYRVVSVLTVLHQDWLNGKEYKCKVSNKALPAPIEKTISKAKGQPREPQVYTLPPSREEMTKNQVSLTCLVKGFYPSDIAVEWESNGQPENNYKTTPPVLDSDGSFFLYSKLTVDKSRWQQGNVFSCSVMHEALHNHYTQKSLSLSPGK

SEQ ID NO: 42 - DNA, 702 bp, synthetic construct
  misc_feature 1..702: note = Humanized Antibody
  source 1..702: mol_type = other DNA
atggtgctgcagacccaggtgttcatctccctgctgctgtggatctccggcgcctacggcgacatccagatgacccagagcccttccagcctgtccgcttccgtgggcgacagagtgaccatcacctgtcaggcctccgaggacatctactccggcctggcctggtatcagcagaagcccggcaagtcccccaagctgctgatctacggcgctggatctctgcaggacggcgtgccctctagattctccggctctggatccggcacccactacaccctgaccatctccagcctgcagcccgaggacttcgctacctacttctgtcagcaaggcctgaagttccccctgaccttcggccagggcaccaaggtggaaatcaagcggaccgtggccgctccctccgtgtttatcttcccaccctccgacgagcagctgaagtccggcacagcttctgtcgtgtgcctgctgaacaacttctacccccgcgaggccaaggtgcagtggaaggtggacaacgccctgcagtccggcaactcccaggaatccgtgaccgagcaggactccaaggacagcacctactccctgtcctctaccctgaccctgtccaaggccgactacgagaagcacaaggtgtacgcctgcgaagtgacccaccagggcctgtctagccccgtgaccaagtctttcaaccggggcgagtgc

SEQ ID NO: 43 - protein, 234 aa, synthetic construct
  REGION 1..234: note = Humanized Antibody
MVLQTQVFISLLLWISGAYGDIQMTQSPSSLSASVGDRVTITCQASEDIYSGLAWYQQKPGKSPKLLIYGAGSLQDGVPSRFSGSGSGTHYTLTISSLQPEDFATYFCQQGLKFPLTFGQGTKVEIKRTVAAPSVFIFPPSDEQLKSGTASVVCLLNNFYPREAKVQWKVDNALQSGNSQESVTEQDSKDSTYSLSSTLTLSKADYEKHKVYACEVTHQGLSSPVTKSFNRGEC

SEQ ID NO: 44 - DNA, 34 bp, synthetic construct
  misc_feature 1..34: note = Primer F
  source 1..34: mol_type = other DNA
cacggcaacctgctggagcggctgctgggggagg

SEQ ID NO: 45 - DNA, 24 bp, synthetic construct
  misc_feature 1..24: note = Primer R
  source 1..24: mol_type = other DNA
caggctgttcccagacaggtccag

SEQ ID NO: 46 - protein, 10 aa, Rattus rattus
  REGION 1..10: note = 151D antibody CDRH1
GFTFSNYYMA

SEQ ID NO: 47 - protein, 10 aa, Rattus rattus
  REGION 1..10: note = 151D antibody CDRH2
SIGTVGGNTY

SEQ ID NO: 48 - protein, 8 aa, Rattus rattus
  REGION 1..8: note = 151D antibody CDRH3
EDYGGFPH

SEQ ID NO: 49 - protein, 11 aa, Rattus rattus
  REGION 1..11: note = 151D antibody CDRL1
KASQNVGTNVD

SEQ ID NO: 50 - protein, 7 aa, Rattus rattus
  REGION 1..7: note = 151D antibody CDRL2
GASNRYT

SEQ ID NO: 51 - protein, 9 aa, Rattus rattus
  REGION 1..9: note = 151D antibody CDRL3
LQYKYNPYT

SEQ ID NO: 52 - protein, 10 aa, Rattus rattus
  REGION 1..10: note = 198D antibody CDRH1
GFSLTSFHVS

SEQ ID NO: 53 - protein, 9 aa, Rattus rattus
  REGION 1..9: note = 198D antibody CDRH2
TISSGGGTY

SEQ ID NO: 54 - protein, 12 aa, Rattus rattus
  REGION 1..12: note = 198D antibody CDRH3
ISGWGHYYVMDV

SEQ ID NO: 55 - protein, 11 aa, Rattus rattus
  REGION 1..11: note = 198D antibody CDRL1
QASEDIYSGLA

SEQ ID NO: 56 - protein, 7 aa, Rattus rattus
  REGION 1..7: note = 198D antibody CDRL2
GAGSLQD

SEQ ID NO: 57 - protein, 9 aa, Rattus rattus
  REGION 1..9: note = 198D antibody CDRL3
QQGLKFPLT